European Patent Specification EP 3 788 032 B1, published January 24, 2024. Title: COMPOUNDS COMPRISING A LINKER FOR INCREASING TRANSCYCLOOCTENE STABILITY. Applicant: Tagworks Pharmaceuticals B.V. The sequence listing filed with the application follows.

SEQUENCE LISTING (1 sequence)

SEQ ID NO: 1 - protein, 234 aa, Artificial Sequence
  TAG72-binding diabody derived from the CC49 antibody
SVQLQQSDAELVKPGASVKISCKASGYTFTDHAIHWVKQNPEQGLEWIGYFSPGNDDFKYNERFKGKATLTADKSSSTAYLQLNSLTSEDSAVYFCTRSLNMAYWGQGTSVTVSSGGGGSDIVMTQSCSSCPVSVGEKVTLSCKSSQSLLYSGNQKNYLAWYQQKPGQSPKLLIYWASTRESGVPDRFTGSGSGTDFTLSISSVETEDLAVYYCQQYYSYPLTFGAGTKLVLKR